European Patent Application EP 4 527 849 A1, published March 26, 2025. Title: HLA-independent antigen binders, such as T-cell receptors, against PD-L1. Applicant: Universitätsmedizin der Johannes Gutenberg-Universität Mainz. Application EP. The sequence listing filed with the application follows.

SEQUENCE LISTING (7 sequences)

SEQ ID NO: 1 - protein, 603 aa, synthetic construct
MGPQLLGYVVLCLLGAGPLEAQVTQNPRYLITVTGKKLTVTCSQNMNHEYMSWYRQDPGLGLRQIYYSMNVEVTDKGDVPEGYKVSRKEKRNFPLILESPSPNQTSLYFCASSLSPAPPSIWSYNEQFFGPGTRLTVLEDLRNVTPPKVSLFEPSKAEIANKQKATLVCLARGFFPDHVELSWWVNGKEVHSGVCTDPQAYKESNYSYCLSSRLRVSATFWHNPRNHFRCQVQFHGLSEEDKWPEGSPKPVTQNISAEAWGRADCGITSASYHQGVLSATILYEILLGKATLYAVLVSGLVLMAMVKKKNSGSGATNFSLLKQAGDVEENPGPMLLLLVPAFQVIFTLGGTRAQSVTQLDSQVPVFEEAPVELRCNYSSSVSVYLFWYVQYPNQGLQLLLKYLSGSTLVKGINGFEAEFNKSQTSFHLRKPSVHISDTAEYFCAVSKLAGRRALTFGSGTRLQVQPNIQNPEPAVYQLKDPRSQDSTLCLFTDFDSQINVPKTMESGTFITDKCVLDMKAMDSKSNGAIAWSNQTSFTCQDIFKETNATYPSSDVPCDATLTEKSFETDMNLNFQNLSVMGLRILLLKVAGFNLLMTLRLWSS

SEQ ID NO: 2 - DNA, 1815 bp, synthetic construct
  source 1..1815: mol_type = other DNA
atgggcccccagctccttggctatgtggtcctttgccttctaggagcaggccccctggaagcccaagtgacccagaacccaagatacctcatcacagtgactggaaagaagttaacagtgacttgttctcagaatatgaaccatgagtatatgtcctggtatcgacaagacccagggctgggcttaaggcagatctactattcaatgaatgttgaggtgactgataagggagatgttcctgaagggtacaaagtctctcgaaaagagaagaggaatttccccctgatcctggagtcgcccagccccaaccagacctctctgtacttctgtgccagcagtttatcccccgcccctcctagcatctggtcctacaatgagcagttcttcgggccagggacacgcctcaccgtgctagaggacctgcggaacgtgaccccccccaaggtgtccctgttcgagcccagcaaggccgagatcgccaacaagcagaaagccacactggtgtgcctcgccaggggcttcttccccgaccacgtggagctgtcttggtgggtgaacggcaaagaggtgcacagcggcgtctgcaccgaccctcaggcctacaaagagagcaactacagctactgcctgtcctcccggctgcgggtgtccgccaccttctggcacaacccccggaaccacttccggtgccaggtgcagttccacggcctgagcgaagaggacaagtggcccgagggcagccccaagcccgtgacccagaacatctccgccgaggcctggggcagagccgactgcggcatcaccagcgccagctaccaccagggcgtgctgtctgccaccatcctgtacgagatcctgctgggcaaggccacactgtacgccgtgctggtgtccggcctggtgctgatggccatggtgaagaaaaagaattctggaagcggagctactaacttcagcctgctgaagcaggctggagacgtggaggagaaccctggacctatgctcctgctgctcgtcccagcgttccaggtgatttttaccctgggaggaaccagagcccagtctgtgacccagcttgacagccaagtccctgtctttgaagaagcccctgtggagctgaggtgcaactactcatcgtctgtttcagtgtatctcttctggtatgtgcaataccccaaccaaggactccagcttctcctgaagtatttatcaggatccaccctggttaaaggcatcaacggttttgaggctgaatttaacaagagtcaaacttccttccacttgaggaaaccctcagtccatataagcgacacggctgagtacttctgtgctgtgagtaaattggcgggcaggagagcacttacttttgggagtggaacaagactccaagtgcaaccaaatatccagaaccctgagcccgccgtgtaccagctgaaggaccccagaagccaggacagcaccctgtgcctgttcaccgacttcgacagccagatcaacgtgcccaagaccatggaaagcggcaccttcatcaccgataagtgcgtgctggacatgaaggccatggacagcaagtccaacggcgccattgcctggtccaaccagaccagcttcacatgccaggacatcttcaaagagacaaacgccacctaccccagcagcgacgtgccctgcgacgccaccctgaccgagaagagcttcgagacagacatgaacctgaacttccagaacctgagcgtgatgggcctgagaatcctgctgctgaaagtggccggcttcaacctgctgatgaccctgcggctgtggagcagctagtaa

SEQ ID NO: 3 - protein, 601 aa, synthetic construct
MDTWLVCWAIFSLLKAGLTEPEVTQTPSHQVTQMGQEVILRCVPISNHLYFYWYRQILGQKVEFLVSFYNNEISEKSEIFDDQFSVERPDGSNFTLKIRSTKLEDSAMYFCASSLRLGWIPGNEQFFGPGTRLTVLEDLRNVTPPKVSLFEPSKAEIANKQKATLVCLARGFFPDHVELSWWVNGKEVHSGVCTDPQAYKESNYSYCLSSRLRVSATFWHNPRNHFRCQVQFHGLSEEDKWPEGSPKPVTQNISAEAWGRADCGITSASYHQGVLSATILYEILLGKATLYAVLVSGLVLMAMVKKKNSGSGATNFSLLKQAGDVEENPGPMLLELIPLLGIHFVLRTARAQSVTQPDIHITVSEGASLELRCNYSYGATPYLFWYVQSPGQGLQLLLKYFSGDTLVQGIKGFEAEFKRSQSSFNLRKPSVHWSDAAEYFCAVGFMDSSYKLIFGSGTRLLVRPDIQNPEPAVYQLKDPRSQDSTLCLFTDFDSQINVPKTMESGTFITDKCVLDMKAMDSKSNGAIAWSNQTSFTCQDIFKETNATYPSSDVPCDATLTEKSFETDMNLNFQNLSVMGLRILLLKVAGFNLLMTLRLWSS

SEQ ID NO: 4 - DNA, 1809 bp, synthetic construct
  source 1..1809: mol_type = other DNA
atggatacctggctcgtatgctgggcaatttttagtctcttgaaagcaggactcacagaacctgaagtcacccagactcccagccatcaggtcacacagatgggacaggaagtgatcttgcgctgtgtccccatctctaatcacttatacttctattggtacagacaaatcttggggcagaaagtcgagtttctggtttccttttataataatgaaatctcagagaagtctgaaatattcgatgatcaattctcagttgaaaggcctgatggatcaaatttcactctgaagatccggtccacaaagctggaggactcagccatgtacttctgtgccagcagtcttcgactaggatggatacccggcaatgagcagttcttcgggccagggacgcgactcaccgtgctagaggacctgcggaacgtgaccccccccaaggtgtccctgttcgagcccagcaaggccgagatcgccaacaagcagaaagccacactggtgtgcctcgccaggggcttcttccccgaccacgtggagctgtcttggtgggtgaacggcaaagaggtgcacagcggcgtctgcaccgaccctcaggcctacaaagagagcaactacagctactgcctgtcctcccggctgcgggtgtccgccaccttctggcacaacccccggaaccacttccggtgccaggtgcagttccacggcctgagcgaagaggacaagtggcccgagggcagccccaagcccgtgacccagaacatctccgccgaggcctggggcagagccgactgcggcatcaccagcgccagctaccaccagggcgtgctgtctgccaccatcctgtacgagatcctgctgggcaaggccacactgtacgccgtgctggtgtccggcctggtgctgatggccatggtgaagaaaaagaattctggaagcggagctactaacttcagcctgctgaagcaggctggagacgtggaggagaaccctggacctatgctcctggagcttatcccactgctggggatacattttgtcctgagaactgccagagcccagtcagtgacccagcctgacatccacatcactgtctctgaaggagcctcactggagttgagatgtaactattcctatggggcaacaccttatctcttctggtatgtccagtcccccggccaaggcctccagctgctcctgaagtacttttcaggagacactctggttcaaggcattaaaggctttgaggctgaatttaagaggagtcaatcttccttcaacctgaggaaaccctctgtgcattggagtgatgctgctgagtacttctgtgctgtgggttttatggatagcagctataaattgatcttcgggagtgggaccagactgctggtcaggcctgatatccagaaccctgagcccgccgtgtaccagctgaaggaccccagaagccaggacagcaccctgtgcctgttcaccgacttcgacagccagatcaacgtgcccaagaccatggaaagcggcaccttcatcaccgataagtgcgtgctggacatgaaggccatggacagcaagtccaacggcgccattgcctggtccaaccagaccagcttcacatgccaggacatcttcaaagagacaaacgccacctaccccagcagcgacgtgccctgcgacgccaccctgaccgagaagagcttcgagacagacatgaacctgaacttccagaacctgagcgtgatgggcctgagaatcctgctgctgaaagtggccggcttcaacctgctgatgaccctgcggctgtggagcagctagtaa

SEQ ID NO: 5 - protein, 610 aa, synthetic construct
MATRLLCCVVLCLLGEELIDARVTQTPRHKVTEMGQEVTMRCQPILGHNTVFWYRQTMMQGLELLAYFRNRAPLDDSGMPKDRFSAEMPDATLATLKIQPSEPRDSAVYFCASGLAPFSREVSYEQYFGPGTRLTVTEDLRNVTPPKVSLFEPSKAEIANKQKATLVCLARGFFPDHVELSWWVNGKEVHSGVCTDPQAYKESNYSYCLSSRLRVSATFWHNPRNHFRCQVQFHGLSEEDKWPEGSPKPVTQNISAEAWGRADCGITSASYHQGVLSATILYEILLGKATLYAVLVSGLVLMAMVKKKNSGSGATNFSLLKQAGDVEENPGPMAMLLGASVLILWLQPDWVNSQQKNDDQQVKQNSPSLSVQEGRISILNCDYTNSMFDYFLWYKKYPAEGPTFLISISSIKDKNEDGRFTVFLNKSAKHLSLHIVPSQPGDSAVYFCAAKAGRETSGSRLTFGEGTQLTVNPDIQNPEPAVYQLKDPRSQDSTLCLFTDFDSQINVPKTMESGTFITDKCVLDMKAMDSKSNGAIAWSNQTSFTCQDIFKETNATYPSSDVPCDATLTEKSFETDMNLNFQNLSVMGLRILLLKVAGFNLLMTLRLWSS

SEQ ID NO: 6 - DNA, 1836 bp, synthetic construct
  source 1..1836: mol_type = other DNA
atggccaccaggctcctctgctgtgtggttctttgtctcctgggagaagagcttatagatgctagagtcacccagacaccaaggcacaaggtgacagagatgggacaagaagtaacaatgagatgtcagccaattttaggccacaatactgttttctggtacagacagaccatgatgcaaggactggagttgctggcttacttccgcaaccgggctcctctagatgattcggggatgccgaaggatcgattctcagcagagatgcctgatgcaactttagccactctgaagatccagccctcagaacccagggactcagctgtgtatttttgtgctagtggtttggcccccttttcgcgggaggtttcctacgagcagtacttcgggccgggcaccaggctcacggtcacagaggacctgcggaacgtgaccccccccaaggtgtccctgttcgagcccagcaaggccgagatcgccaacaagcagaaagccacactggtgtgcctcgccaggggcttcttccccgaccacgtggagctgtcttggtgggtgaacggcaaagaggtgcacagcggcgtctgcaccgaccctcaggcctacaaagagagcaactacagctactgcctgtcctcccggctgcgggtgtccgccaccttctggcacaacccccggaaccacttccggtgccaggtgcagttccacggcctgagcgaagaggacaagtggcccgagggcagccccaagcccgtgacccagaacatctccgccgaggcctggggcagagccgactgcggcatcaccagcgccagctaccaccagggcgtgctgtctgccaccatcctgtacgagatcctgctgggcaaggccacactgtacgccgtgctggtgtccggcctggtgctgatggccatggtgaagaaaaagaattctggaagcggagctactaacttcagcctgctgaagcaggctggagacgtggaggagaaccctggacctatggccatgctcctgggggcatcagtgctgattctgtggcttcagccagactgggtaaacagtcaacagaagaatgatgaccagcaagttaagcaaaattcaccatccctgagcgtccaggaaggaagaatttctattctgaactgtgactatactaacagcatgtttgattatttcctatggtacaaaaaataccctgctgaaggtcctacattcctgatatctataagttccattaaggataaaaatgaagatggaagattcactgtcttcttaaacaaaagtgccaagcacctctctctgcacattgtgccctcccagcctggagactctgcagtgtacttctgtgcagcaaaggccggtcgggaaaccagtggctctaggttgacctttggggaaggaacacagctcacagtgaatcctgatatccagaaccctgagcccgccgtgtaccagctgaaggaccccagaagccaggacagcaccctgtgcctgttcaccgacttcgacagccagatcaacgtgcccaagaccatggaaagcggcaccttcatcaccgataagtgcgtgctggacatgaaggccatggacagcaagtccaacggcgccattgcctggtccaaccagaccagcttcacatgccaggacatcttcaaagagacaaacgccacctaccccagcagcgacgtgccctgcgacgccaccctgaccgagaagagcttcgagacagacatgaacctgaacttccagaacctgagcgtgatgggcctgagaatcctgctgctgaaagtggccggcttcaacctgctgatgaccctgcggctgtggagcagctagtaa

SEQ ID NO: 7 - protein, 290 aa, Homo sapiens
MRIFAVFIFMTYWHLLNAFTVTVPKDLYVVEYGSNMTIECKFPVEKQLDLAALIVYWEMEDKNIIQFVHGEEDLKVQHSSYRQRARLLKDQLSLGNAALQITDVKLQDAGVYRCMISYGGADYKRITVKVNAPYNKINQRILVVDPVTSEHELTCQAEGYPKAEVIWTSSDHQVLSGKTTTTNSKREEKLFNVTSTLRINTTTNEIFYCTFRRLDPEENHTAELVIPELPLAHPPNERTHLVILGAILLCLGVALTFIFRLRKGRMMDVKKCGIQDTNSKKQSDTHLEET